European Patent Specification EP 3 943 614 B1, published February 21, 2024. Title: Novel Probe Set for Isothermal One-pot Reaction and Uses Thereof. Applicant: POSTECH ACADEMY-INDUSTRY FOUNDATION. The sequence listing filed with the application follows.

SEQUENCE LISTING (20 sequences)

SEQ ID NO: 1 - DNA, 87 bp, Artificial Sequence
  promoter probe
ttctccttgtttcattttgagttctgcagccctatagtgagtcgtattaggatccacaacaggatcctaatacgactcactataggg

SEQ ID NO: 2 - DNA, 61 bp, Artificial Sequence
  reporter probe
gggatccattcgttacctggctctcgccagtcgggatccaccacccaatttgtctgccagt

SEQ ID NO: 3 - DNA, 82 bp, Artificial Sequence
  promoter probe
ttcttgtgcgccaacctgtaccctatagtgagtcgtattaatttcgcgacaacacgcgaaattaatacgactcactataggg

SEQ ID NO: 4 - DNA, 59 bp, Artificial Sequence
  reporter probe
ggatccattcgttacctggctctcgccagtcgggatcccttctcaacaatcggcacata

SEQ ID NO: 5 - DNA, 82 bp, Artificial Sequence
  promoter probe
tcaactccccaacgccttttccctatagtgagtcgtattaatttcgcgacaacacgcgaaattaatacgactcactataggg

SEQ ID NO: 6 - DNA, 58 bp, Artificial Sequence
  reporter probe
ggatccattcgttacctggctctcgccagtcgggatcccgcaccgctatttgactccc

SEQ ID NO: 7 - DNA, 82 bp, Artificial Sequence
  promoter probe
aagaggaactgaatcgcgcgccctatagtgagtcgtattaatttcgcgacaacacgcgaaattaatacgactcactataggg

SEQ ID NO: 8 - DNA, 58 bp, Artificial Sequence
  reporter probe
ggatccattcgttacctggctctcgccagtcgggatccgagctcggggcgattatgtg

SEQ ID NO: 9 - DNA, 82 bp, Artificial Sequence
  promoter probe
tcccctgctcattgctatggccctatagtgagtcgtattaatttcgcgacaacacgcgaaattaatacgactcactataggg

SEQ ID NO: 10 - DNA, 58 bp, Artificial Sequence
  reporter probe
ggatccattcgttacctggctctcgccagtcgggatcctttgtctgcagcgtatccac

SEQ ID NO: 11 - DNA, 83 bp, Artificial Sequence
  promoter probe
ttccacaacatacaccccctcccctatagtgagtcgtattaatttcgcgacaacacgcgaaattaatacgactcactataggg

SEQ ID NO: 12 - DNA, 88 bp, Artificial Sequence
  reporter probe
gtatgtgggagacggtcgggtccagatattcgtatctgtcgagtagagtgtgggctcccacatacgggcgataaactctagtatgcca

SEQ ID NO: 13 - DNA, 86 bp, Artificial Sequence
  promoter probe
gttccacctggtttaacatatagtccctatagtgagtcgtattaatttcgcgacaacacgcgaaattaatacgactcactataggg

SEQ ID NO: 14 - DNA, 56 bp, Artificial Sequence
  reporter probe
ggatccattcgttacctggctctcgccagtcgggatccgtggcatctcctgatgag

SEQ ID NO: 15 - DNA, 87 bp, Artificial Sequence
  promoter probe
acactattagcataagcagttgtggccctatagtgagtcgtattaatttcgcgacaacacgcgaaattaatacgactcactataggg

SEQ ID NO: 16 - DNA, 61 bp, Artificial Sequence
  reporter probe
ggatccattcgttacctggctctcgccagtcgggatcctgacagcttgacaaatgttaaaa

SEQ ID NO: 17 - DNA, 88 bp, Artificial Sequence
  promoter probe
aacactattagcataagcagttgtggccctatagtgagtcgtattaatttcgcgacaacacgcgaaattaatacgactcactataggg

SEQ ID NO: 18 - DNA, 88 bp, Artificial Sequence
  reporter probe
gtatgtgggagacggtcgggtccagatattcgtatctgtcgagtagagtgtgggctcccacatacgtgacagcttgacaaatgttaaa

SEQ ID NO: 19 - DNA, 90 bp, Artificial Sequence
  promoter probe
tttcactcaatacttgagcacactcattccctatagtgagtcgtattaatttcgcgacaacacgcgaaattaatacgactcactataggg

SEQ ID NO: 20 - DNA, 84 bp, Artificial Sequence
  reporter probe
gtatgtgggagacggtcgggtccagatattcgtatctgtcgagtagagtgtgggctcccacatactaaccgccacacatgacca